European Patent Application EP 4 397 774 A2, published July 10, 2024. Title: METHODS FOR BARCODING NUCLEIC ACID MOLECULES FROM INDIVIDUAL CELLS OR CELL POPULATIONS. Applicant: 10x Genomics, Inc. Application EP 24163869.1, filed October 18, 2017. The sequence listing filed with the application follows.

SEQUENCE LISTING (170 sequences)

SEQ ID NO: 1 - DNA, 13 bp, synthetic construct
  source 1..13: mol_type = other DNA
tttcttatatggg

SEQ ID NO: 2 - DNA, 23 bp, synthetic construct
  source 1..23: mol_type = other DNA
aaatcaaatctttcttatatggg

SEQ ID NO: 3 - DNA, 33 bp, synthetic construct
  source 1..33: mol_type = other DNA
acaaacaaataaatcaaatctttcttatatggg

SEQ ID NO: 4 - DNA, 13 bp, synthetic construct
  source 1..13: mol_type = other DNA
gaaatttaaaggg

SEQ ID NO: 5 - DNA, 23 bp, synthetic construct
  source 1..23: mol_type = other DNA
cactctacatgaaatttaaaggg

SEQ ID NO: 6 - DNA, 33 bp, synthetic construct
  source 1..33: mol_type = other DNA
ccaaagttgtcactctacatgaaatttaaaggg

SEQ ID NO: 7 - DNA, 13 bp, synthetic construct
  source 1..13: mol_type = other DNA
atatatataaggg

SEQ ID NO: 8 - DNA, 23 bp, synthetic construct
  source 1..23: mol_type = other DNA
atatatatatatatatataaggg

SEQ ID NO: 9 - DNA, 33 bp, synthetic construct
  source 1..33: mol_type = other DNA
atatatatatatatatatatatatatataaggg

SEQ ID NO: 10 - DNA, 30 bp, synthetic construct
  source 1..30: mol_type = other DNA
gccggccgccccggcggccgccgcgcggcc

SEQ ID NO: 11 - DNA, 30 bp, synthetic construct
  source 1..30: mol_type = other DNA
gccgccggcgcccgccccccggccggggcc

SEQ ID NO: 12 - DNA, 30 bp, synthetic construct
  source 1..30: mol_type = other DNA
gcgcgcgcgcgcgccgcccccgccgctccc

SEQ ID NO: 13 - DNA, 30 bp, synthetic construct
  source 1..30: mol_type = other DNA
ggggcgcgccgcgccgccgccgggctcccc

SEQ ID NO: 14 - DNA, 30 bp, synthetic construct
  source 1..30: mol_type = other DNA
gccgccgccaccgccgccgccgccgccgcc

SEQ ID NO: 15 - DNA, 30 bp, synthetic construct
  source 1..30: mol_type = other DNA
gccccgccccgccgcccgccgaccgccgcc

SEQ ID NO: 16 - DNA, 30 bp, synthetic construct
  source 1..30: mol_type = other DNA
gcggcccctccgccgcctgccgccgccgcc

SEQ ID NO: 17 - DNA, 30 bp, synthetic construct
  source 1..30: mol_type = other DNA
ggagcgggtcgcgcccggccgggcgggcgc

SEQ ID NO: 18 - DNA, 30 bp, synthetic construct
  source 1..30: mol_type = other DNA
gccccgccccccgacccgcgcgcggcaccc

SEQ ID NO: 19 - DNA, 30 bp, synthetic construct
  source 1..30: mol_type = other DNA
ggcggcccgcagggccgcggaccccgcccc

SEQ ID NO: 20 - DNA, 30 bp, synthetic construct
  source 1..30: mol_type = other DNA
ggcggggcacgcgccctcccgcggcggggc

SEQ ID NO: 21 - DNA, 30 bp, synthetic construct
  source 1..30: mol_type = other DNA
gccagggccgtgggccgaccccggcggggc

SEQ ID NO: 22 - DNA, 30 bp, synthetic construct
  source 1..30: mol_type = other DNA
gtcccccgccgaccccacccccggccccgc

SEQ ID NO: 23 - DNA, 30 bp, synthetic construct
  source 1..30: mol_type = other DNA
ggctcgcctcgcggcggaccgcccgcccgc

SEQ ID NO: 24 - DNA, 30 bp, synthetic construct
  source 1..30: mol_type = other DNA
gacccgggcgcgcgccggccgctaccggcc

SEQ ID NO: 25 - DNA, 30 bp, synthetic construct
  source 1..30: mol_type = other DNA
gcgcgcctcgtccagccgcggcgcgcgccc

SEQ ID NO: 26 - DNA, 30 bp, synthetic construct
  source 1..30: mol_type = other DNA
gcgccgtgggaggggtggcccggccccccc

SEQ ID NO: 27 - DNA, 30 bp, synthetic construct
  source 1..30: mol_type = other DNA
gggccccccgagccaccttccccgccgggc

SEQ ID NO: 28 - DNA, 30 bp, synthetic construct
  source 1..30: mol_type = other DNA
ggcggctccacccgggcccgcgccctaggc

SEQ ID NO: 29 - DNA, 30 bp, synthetic construct
  source 1..30: mol_type = other DNA
ggcgcggggtggggagggagcgagcggcgc

SEQ ID NO: 30 - DNA, 30 bp, synthetic construct
  source 1..30: mol_type = other DNA
gctaggcgccggccgaggcgaggcgcgcgc

SEQ ID NO: 31 - DNA, 30 bp, synthetic construct
  source 1..30: mol_type = other DNA
gtcccgcgccccgcggggcggggattcggc

SEQ ID NO: 32 - DNA, 30 bp, synthetic construct
  source 1..30: mol_type = other DNA
ggggcggccgcctttccggccgcgccccgt

SEQ ID NO: 33 - DNA, 30 bp, synthetic construct
  source 1..30: mol_type = other DNA
acctccccggcgcggcgggcgagacgggcc

SEQ ID NO: 34 - DNA, 30 bp, synthetic construct
  source 1..30: mol_type = other DNA
gatccgccgggccgccgacacggccggacc

SEQ ID NO: 35 - DNA, 30 bp, synthetic construct
  source 1..30: mol_type = other DNA
gccgaccccgtgcgctcgctccgccgtccc

SEQ ID NO: 36 - DNA, 30 bp, synthetic construct
  source 1..30: mol_type = other DNA
gcgcggcgacgggtctcgctccctcggccc

SEQ ID NO: 37 - DNA, 30 bp, synthetic construct
  source 1..30: mol_type = other DNA
gcccggctcgcgtccagagtccgcgccgcc

SEQ ID NO: 38 - DNA, 30 bp, synthetic construct
  source 1..30: mol_type = other DNA
tccccggggctcccgccggcttctccggga

SEQ ID NO: 39 - DNA, 30 bp, synthetic construct
  source 1..30: mol_type = other DNA
acctcggccggcgagcgcgccggccttcac

SEQ ID NO: 40 - DNA, 30 bp, synthetic construct
  source 1..30: mol_type = other DNA
acgcccggctccacgccagcgagccgggct

SEQ ID NO: 41 - DNA, 30 bp, synthetic construct
  source 1..30: mol_type = other DNA
gctcaccggacgccgccggaaccgcgacgc

SEQ ID NO: 42 - DNA, 30 bp, synthetic construct
  source 1..30: mol_type = other DNA
tcgcccgtcccttcggaacggcgctcgccc

SEQ ID NO: 43 - DNA, 30 bp, synthetic construct
  source 1..30: mol_type = other DNA
ggggtgcgtcgggtctgcgagagcgccagc

SEQ ID NO: 44 - DNA, 30 bp, synthetic construct
  source 1..30: mol_type = other DNA
ggccaaccgaggctccgcggcgctgccgta

SEQ ID NO: 45 - DNA, 30 bp, synthetic construct
  source 1..30: mol_type = other DNA
gttacccgcgcctgccggcgtagggtaggc

SEQ ID NO: 46 - DNA, 30 bp, synthetic construct
  source 1..30: mol_type = other DNA
gcgtcaacacccgccgcgggccttcgcgat

SEQ ID NO: 47 - DNA, 30 bp, synthetic construct
  source 1..30: mol_type = other DNA
agctgcggtatccaggcggctcgggcctgc

SEQ ID NO: 48 - DNA, 30 bp, synthetic construct
  source 1..30: mol_type = other DNA
gcgtcggcatcgggcgccttaacccggcgt

SEQ ID NO: 49 - DNA, 30 bp, synthetic construct
  source 1..30: mol_type = other DNA
gggaataacgccgccgcatcgccggtcggc

SEQ ID NO: 50 - DNA, 30 bp, synthetic construct
  source 1..30: mol_type = other DNA
gcggcgcaatacgaatgcccccggccgtcc

SEQ ID NO: 51 - DNA, 30 bp, synthetic construct
  source 1..30: mol_type = other DNA
tgctgcggatatgggtacggcccggcgcga

SEQ ID NO: 52 - DNA, 30 bp, synthetic construct
  source 1..30: mol_type = other DNA
gggcagacgttcgaatgggtcgtcgccgcc

SEQ ID NO: 53 - DNA, 30 bp, synthetic construct
  source 1..30: mol_type = other DNA
gccgcaggctccactcctggtggtgccctt

SEQ ID NO: 54 - DNA, 30 bp, synthetic construct
  source 1..30: mol_type = other DNA
accgcggctgctggcaccagacttgccctc

SEQ ID NO: 55 - DNA, 30 bp, synthetic construct
  source 1..30: mol_type = other DNA
gggtcgggagtgggtaatttgcgcgcctgc

SEQ ID NO: 56 - DNA, 30 bp, synthetic construct
  source 1..30: mol_type = other DNA
agcgggtcgccacgtctgatctgaggtcgc

SEQ ID NO: 57 - DNA, 30 bp, synthetic construct
  source 1..30: mol_type = other DNA
ttccccgctgattccgccaagcccgttccc

SEQ ID NO: 58 - DNA, 30 bp, synthetic construct
  source 1..30: mol_type = other DNA
tgcacgtcaggaccgctacggacctccacc

SEQ ID NO: 59 - DNA, 30 bp, synthetic construct
  source 1..30: mol_type = other DNA
agcggattccgacttccatggccaccgtcc

SEQ ID NO: 60 - DNA, 30 bp, synthetic construct
  source 1..30: mol_type = other DNA
agcttcgccccattggctcctcagccaagc

SEQ ID NO: 61 - DNA, 30 bp, synthetic construct
  source 1..30: mol_type = other DNA
gatcgcagcgagggagctgctctgctacgt

SEQ ID NO: 62 - DNA, 30 bp, synthetic construct
  source 1..30: mol_type = other DNA
gaacggccatgcaccaccacccacggaatc

SEQ ID NO: 63 - DNA, 30 bp, synthetic construct
  source 1..30: mol_type = other DNA
tctcgggtggctgaacgccacttgtccctc

SEQ ID NO: 64 - DNA, 30 bp, synthetic construct
  source 1..30: mol_type = other DNA
gggtcagcgcccgtcggcatgtattagctc

SEQ ID NO: 65 - DNA, 30 bp, synthetic construct
  source 1..30: mol_type = other DNA
tcctccctgagctcgccttaggacacctgc

SEQ ID NO: 66 - DNA, 30 bp, synthetic construct
  source 1..30: mol_type = other DNA
ggaatcgaaccctgattccccgtcacccgt

SEQ ID NO: 67 - DNA, 30 bp, synthetic construct
  source 1..30: mol_type = other DNA
acgggcggtgtgtacaaagggcagggactt

SEQ ID NO: 68 - DNA, 30 bp, synthetic construct
  source 1..30: mol_type = other DNA
tacggatccggcttgccgacttcccttacc

SEQ ID NO: 69 - DNA, 30 bp, synthetic construct
  source 1..30: mol_type = other DNA
accggccgtgcgtacttagacatgcatggc

SEQ ID NO: 70 - DNA, 30 bp, synthetic construct
  source 1..30: mol_type = other DNA
gtcatagttactcccgccgtttacccgcgc

SEQ ID NO: 71 - DNA, 30 bp, synthetic construct
  source 1..30: mol_type = other DNA
gatccttccgcaggttcacctacggaaacc

SEQ ID NO: 72 - DNA, 30 bp, synthetic construct
  source 1..30: mol_type = other DNA
tcacgacggtctaaacccagctcacgttcc

SEQ ID NO: 73 - DNA, 30 bp, synthetic construct
  source 1..30: mol_type = other DNA
ggccccgctttcacggtctgtattcgtact

SEQ ID NO: 74 - DNA, 30 bp, synthetic construct
  source 1..30: mol_type = other DNA
gtacttgttgactatcggtctcgtgccggt

SEQ ID NO: 75 - DNA, 30 bp, synthetic construct
  source 1..30: mol_type = other DNA
ggaacccttctccacttcggccttcaaagt

SEQ ID NO: 76 - DNA, 30 bp, synthetic construct
  source 1..30: mol_type = other DNA
acccgtttacctcttaacggtttcacgccc

SEQ ID NO: 77 - DNA, 30 bp, synthetic construct
  source 1..30: mol_type = other DNA
gaacctccgactttcgttcttgattaatga

SEQ ID NO: 78 - DNA, 50 bp, synthetic construct
  source 1..50: mol_type = other DNA
gcccccgccggccgccccggcggccgccgcgcggcccctgccgccccgac

SEQ ID NO: 79 - DNA, 50 bp, synthetic construct
  source 1..50: mol_type = other DNA
gcccccgccgccgccgccaccgccgccgccgccgccgccccgacccgcgc

SEQ ID NO: 80 - DNA, 50 bp, synthetic construct
  source 1..50: mol_type = other DNA
ggaccggcccgcggcccctccgccgcctgccgccgccgccgccgcgcgcc

SEQ ID NO: 81 - DNA, 50 bp, synthetic construct
  source 1..50: mol_type = other DNA
gccccgccccgccgcccgccgaccgccgccgcccgaccgctcccgccccc

SEQ ID NO: 82 - DNA, 50 bp, synthetic construct
  source 1..50: mol_type = other DNA
gtccgccccgccccccgacccgcgcgcggcaccccccccgtcgccggggc

SEQ ID NO: 83 - DNA, 50 bp, synthetic construct
  source 1..50: mol_type = other DNA
accccggtcccggcgcgcggcggggcacgcgccctcccgcggcggggcgc

SEQ ID NO: 84 - DNA, 50 bp, synthetic construct
  source 1..50: mol_type = other DNA
ggccccgcccgcccacccccgcacccgccggagcccgccccctccgggga

SEQ ID NO: 85 - DNA, 50 bp, synthetic construct
  source 1..50: mol_type = other DNA
ggcggcccgcagggccgcggaccccgccccgggcccctcgcggggacacc

SEQ ID NO: 86 - DNA, 50 bp, synthetic construct
  source 1..50: mol_type = other DNA
gccgccctccgacgcacaccacacgcgcgcgcgcgcgcgccgcccccgcc

SEQ ID NO: 87 - DNA, 50 bp, synthetic construct
  source 1..50: mol_type = other DNA
ggggcgcgcgcctcgtccagccgcggcgcgcgcccagccccgcttcgcgc

SEQ ID NO: 88 - DNA, 50 bp, synthetic construct
  source 1..50: mol_type = other DNA
agccgccggcgcccgccccccggccggggccggagaggggctgaccgggt

SEQ ID NO: 89 - DNA, 50 bp, synthetic construct
  source 1..50: mol_type = other DNA
gggcggggacgggcggtggctcgcctcgcggcggaccgcccgcccgctcc

SEQ ID NO: 90 - DNA, 50 bp, synthetic construct
  source 1..50: mol_type = other DNA
gggcccggctcgcgtccagagtccgcgccgccgccggccccccgggtccc

SEQ ID NO: 91 - DNA, 50 bp, synthetic construct
  source 1..50: mol_type = other DNA
ggcactgtccccggagcgggtcgcgcccggccgggcgggcgcttggcgcc

SEQ ID NO: 92 - DNA, 50 bp, synthetic construct
  source 1..50: mol_type = other DNA
gcgccgtgggaggggtggcccggcccccccacgaggagacgccggcgcgc

SEQ ID NO: 93 - DNA, 50 bp, synthetic construct
  source 1..50: mol_type = other DNA
tccacctccccggcgcggcgggcgagacgggccggtggtgcgccctcggc

SEQ ID NO: 94 - DNA, 50 bp, synthetic construct
  source 1..50: mol_type = other DNA
tccccgccgggccttcccagccgtcccggagccggtcgcggcgcaccgcc

SEQ ID NO: 95 - DNA, 50 bp, synthetic construct
  source 1..50: mol_type = other DNA
gtcggctgctaggcgccggccgaggcgaggcgcgcgcggaaccgcggccc

SEQ ID NO: 96 - DNA, 50 bp, synthetic construct
  source 1..50: mol_type = other DNA
gggcgcgcgccggccgctaccggcctcacaccgtccacgggctgggcctc

SEQ ID NO: 97 - DNA, 50 bp, synthetic construct
  source 1..50: mol_type = other DNA
gggacgcgcgcgtggccccgagagaacctcccccgggcccgacggcgcga

SEQ ID NO: 98 - DNA, 50 bp, synthetic construct
  source 1..50: mol_type = other DNA
ggcgggaaagatccgccgggccgccgacacggccggacccgccgccgggt

SEQ ID NO: 99 - DNA, 50 bp, synthetic construct
  source 1..50: mol_type = other DNA
gaccgtcttctcagcgctccgccagggccgtgggccgaccccggcggggc

SEQ ID NO: 100 - DNA, 50 bp, synthetic construct
  source 1..50: mol_type = other DNA
agcggcgccggggagcgggtcttccgtacgccacatgtcccgcgccccgc

SEQ ID NO: 101 - DNA, 50 bp, synthetic construct
  source 1..50: mol_type = other DNA
ggctcaccgcagcggccctcctactcgtcgcggcgtagcgtccgcggggc

SEQ ID NO: 102 - DNA, 50 bp, synthetic construct
  source 1..50: mol_type = other DNA
gcgcggcgacgggtctcgctccctcggccccgggattcggcgagtgctgc

SEQ ID NO: 103 - DNA, 50 bp, synthetic construct
  source 1..50: mol_type = other DNA
acctcggccggcgagcgcgccggccttcaccttcattgcgccacggcggc

SEQ ID NO: 104 - DNA, 50 bp, synthetic construct
  source 1..50: mol_type = other DNA
ggccgagggcaacggaggccatcgcccgtcccttcggaacggcgctcgcc

SEQ ID NO: 105 - DNA, 50 bp, synthetic construct
  source 1..50: mol_type = other DNA
gaggccaaccgaggctccgcggcgctgccgtatcgttcgcctgggcggga

SEQ ID NO: 106 - DNA, 50 bp, synthetic construct
  source 1..50: mol_type = other DNA
agctcaccggacgccgccggaaccgcgacgctttccaaggcacgggcccc

SEQ ID NO: 107 - DNA, 50 bp, synthetic construct
  source 1..50: mol_type = other DNA
tcaagacgggtcgggtgggtagccgacgtcgccgccgaccccgtgcgctc

SEQ ID NO: 108 - DNA, 50 bp, synthetic construct
  source 1..50: mol_type = other DNA
tctccccggggctcccgccggcttctccgggatcggtcgcgttaccgcac

SEQ ID NO: 109 - DNA, 50 bp, synthetic construct
  source 1..50: mol_type = other DNA
gctgcccggcgggtcatgggaataacgccgccgcatcgccggtcggcatc

SEQ ID NO: 110 - DNA, 50 bp, synthetic construct
  source 1..50: mol_type = other DNA
gtggcccactaggcactcgcattccacgcccggctccacgccagcgagcc

SEQ ID NO: 111 - DNA, 50 bp, synthetic construct
  source 1..50: mol_type = other DNA
gcgacggccgggtatgggcccgacgctccagcgccatccattttcagggc

SEQ ID NO: 112 - DNA, 50 bp, synthetic construct
  source 1..50: mol_type = other DNA
gggtaggcacacgctgagccagtcagtgtagcgcgcgtgcagccccggac

SEQ ID NO: 113 - DNA, 50 bp, synthetic construct
  source 1..50: mol_type = other DNA
ggggtctgatgagcgtcggcatcgggcgccttaacccggcgttcggttca

SEQ ID NO: 114 - DNA, 50 bp, synthetic construct
  source 1..50: mol_type = other DNA
gcactgggcagaaatcacatcgcgtcaacacccgccgcgggccttcgcga

SEQ ID NO: 115 - DNA, 50 bp, synthetic construct
  source 1..50: mol_type = other DNA
gaggctgttcaccttggagacctgctgcggatatgggtacggcccggcgc

SEQ ID NO: 116 - DNA, 50 bp, synthetic construct
  source 1..50: mol_type = other DNA
tcgtcactacctccccgggtcgggagtgggtaatttgcgcgcctgctgcc

SEQ ID NO: 117 - DNA, 50 bp, synthetic construct
  source 1..50: mol_type = other DNA
gaatggtttagcgccaggttccccacgaacgtgcggtgcgtgacgggcga

SEQ ID NO: 118 - DNA, 50 bp, synthetic construct
  source 1..50: mol_type = other DNA
gcgtcgggtctgcgagagcgccagctatcctgagggaaacttcggaggga

SEQ ID NO: 119 - DNA, 50 bp, synthetic construct
  source 1..50: mol_type = other DNA
acccaggtcggacgaccgatttgcacgtcaggaccgctacggacctccac

SEQ ID NO: 120 - DNA, 50 bp, synthetic construct
  source 1..50: mol_type = other DNA
tcgaaccctgattccccgtcacccgtggtcaccatggtaggcacggcgac

SEQ ID NO: 121 - DNA, 50 bp, synthetic construct
  source 1..50: mol_type = other DNA
ttccccgctgattccgccaagcccgttcccttggctgtggtttcgctgga

SEQ ID NO: 122 - DNA, 50 bp, synthetic construct
  source 1..50: mol_type = other DNA
gcggcgcaatacgaatgcccccggccgtccctcttaatcatggcctcagt

SEQ ID NO: 123 - DNA, 50 bp, synthetic construct
  source 1..50: mol_type = other DNA
gggccgggtgaggtttcccgtgttgagtcaaattaagccgcaggctccac

SEQ ID NO: 124 - DNA, 50 bp, synthetic construct
  source 1..50: mol_type = other DNA
ggtcctattccattattcctagctgcggtatccaggcggctcgggcctgc

SEQ ID NO: 125 - DNA, 50 bp, synthetic construct
  source 1..50: mol_type = other DNA
gctattggagctggaattaccgcggctgctggcaccagacttgccctcca

SEQ ID NO: 126 - DNA, 50 bp, synthetic construct
  source 1..50: mol_type = other DNA
gtcctccctgagctcgccttaggacacctgcgttaccgtttgacaggtgt

SEQ ID NO: 127 - DNA, 50 bp, synthetic construct
  source 1..50: mol_type = other DNA
tcgctccaccaactaagaacggccatgcaccaccacccacggaatcgaga

SEQ ID NO: 128 - DNA, 50 bp, synthetic construct
  source 1..50: mol_type = other DNA
gggctgactttcaatagatcgcagcgagggagctgctctgctacgtacga

SEQ ID NO: 129 - DNA, 50 bp, synthetic construct
  source 1..50: mol_type = other DNA
gttacacactccttagcggattccgacttccatggccaccgtcctgctgt

SEQ ID NO: 130 - DNA, 50 bp, synthetic construct
  source 1..50: mol_type = other DNA
atcccacagatggtagcttcgccccattggctcctcagccaagcacatac

SEQ ID NO: 131 - DNA, 50 bp, synthetic construct
  source 1..50: mol_type = other DNA
gccattcgcagtttcactgtaccggccgtgcgtacttagacatgcatggc

SEQ ID NO: 132 - DNA, 50 bp, synthetic construct
  source 1..50: mol_type = other DNA
ggtagtagcgacgggcggtgtgtacaaagggcagggacttaatcaacgca

SEQ ID NO: 133 - DNA, 50 bp, synthetic construct
  source 1..50: mol_type = other DNA
gcggaccccacccgtttacctcttaacggtttcacgccctcttgaactct

SEQ ID NO: 134 - DNA, 50 bp, synthetic construct
  source 1..50: mol_type = other DNA
ttgaatatttgctactaccaccaagatctgcacctgcggcggctccaccc

SEQ ID NO: 135 - DNA, 50 bp, synthetic construct
  source 1..50: mol_type = other DNA
ttagagccaatccttatcccgaagttacggatccggcttgccgacttccc

SEQ ID NO: 136 - DNA, 50 bp, synthetic construct
  source 1..50: mol_type = other DNA
tcgtgccggtatttagccttagatggagtttaccacccgctttgggctgc

SEQ ID NO: 137 - DNA, 50 bp, synthetic construct
  source 1..50: mol_type = other DNA
ggcatttggctaccttaagagagtcatagttactcccgccgtttacccgc

SEQ ID NO: 138 - DNA, 50 bp, synthetic construct
  source 1..50: mol_type = other DNA
aacctgtctcacgacggtctaaacccagctcacgttccctattagtgggt

SEQ ID NO: 139 - DNA, 50 bp, synthetic construct
  source 1..50: mol_type = other DNA
gggtcagcgcccgtcggcatgtattagctctagaattaccacagttatcc

SEQ ID NO: 140 - DNA, 50 bp, synthetic construct
  source 1..50: mol_type = other DNA
gccccgctttcacggtctgtattcgtactgaaaatcaagatcaagcgagc

SEQ ID NO: 141 - DNA, 50 bp, synthetic construct
  source 1..50: mol_type = other DNA
tcctccgctgactaatatgcttaaattcagcgggtcgccacgtctgatct

SEQ ID NO: 142 - DNA, 50 bp, synthetic construct
  source 1..50: mol_type = other DNA
gttattgctcaatctcgggtggctgaacgccacttgtccctctaagaagt

SEQ ID NO: 143 - DNA, 50 bp, synthetic construct
  source 1..50: mol_type = other DNA
tgagaataggttgagatcgtttcggccccaagacctctaatcattcgctt

SEQ ID NO: 144 - DNA, 50 bp, synthetic construct
  source 1..50: mol_type = other DNA
gtcttcgaacctccgactttcgttcttgattaatgaaaacattcttggca

SEQ ID NO: 145 - DNA, 75 bp, synthetic construct
  misc_feature 1..72: note = DNA
  source 1..75: mol_type = other DNA
  misc_feature 73..75: note = RNA
caagcagaagacggcatacgagatnnnnnngtnnnnnngtgactggagttcagacgtgtgctcttccgatctggg

SEQ ID NO: 146 - DNA, 85 bp, synthetic construct
  misc_feature 1..82: note = DNA
  misc_feature 83..85: note = RNA
  source 1..85: mol_type = other DNA
caagcagaagacggcatacgagatnnnnnnnnnnnnnnnngtnnnnnngtgactggagttcagacgtgtgctcttccgatctggg

SEQ ID NO: 147 - DNA, 79 bp, synthetic construct
  misc_feature 1..76: note = DNA
  misc_feature 77..79: note = RNA
  source 1..79: mol_type = other DNA
aatgatacggcgaccaccgagatctacacnnnnnngtnnnnnnacactctttccctacacgacgctcttccgatctggg

SEQ ID NO: 148 - DNA, 89 bp, synthetic construct
  misc_feature 1..86: note = DNA
  misc_feature 87..89: note = RNA
  source 1..89: mol_type = other DNA
aatgatacggcgaccaccgagatctacacnnnnnnnnnnnnnnnngtnnnnnnacactctttccctacacgacgctcttccgatctggg

SEQ ID NO: 149 - DNA, 39 bp, synthetic construct
  misc_feature 1..36: note = DNA
  misc_feature 37..39: note = RNA
  source 1..39: mol_type = other DNA
ctacacgacgctcttccgatctnnnnnngtnnnnnnggg

SEQ ID NO: 150 - DNA, 49 bp, synthetic construct
  misc_feature 1..46: note = DNA
  misc_feature 47..49: note = RNA
  source 1..49: mol_type = other DNA
ctacacgacgctcttccgatctnnnnnngtnnnnnnnnnnnnnnnnggg

SEQ ID NO: 151 - DNA, 47 bp, synthetic construct
  misc_feature 1..44: note = DNA
  misc_feature 45..47: note = RNA
  source 1..47: mol_type = other DNA
ctacacgacgctcttccgatctnnnnnngtnnnnnnnnnnnnwwggg

SEQ ID NO: 152 - DNA, 49 bp, synthetic construct
  misc_feature 1..46: note = DNA
  misc_feature 47..49: note = RNA
  source 1..49: mol_type = other DNA
ctacacgacgctcttccgatctnnnnnnnnnnnnnnnngtnnnnnnggg

SEQ ID NO: 153 - DNA, 51 bp, synthetic construct
  misc_feature 1..48: note = DNA
  misc_feature 49..51: note = RNA
  source 1..51: mol_type = other DNA
ctacacgacgctcttccgatctnnnnnngtnnnnnnnnnnnnnnnnatggg

SEQ ID NO: 154 - DNA, 53 bp, synthetic construct
  misc_feature 1..50: note = DNA
  misc_feature 51..53: note = RNA
  source 1..53: mol_type = other DNA
ctacacgacgctcttccgatctnnnnnngtnnnnnnnnnnnnnnnnacatggg

SEQ ID NO: 155 - DNA, 55 bp, synthetic construct
  misc_feature 1..52: note = DNA
  misc_feature 53..55: note = RNA
  source 1..55: mol_type = other DNA
ctacacgacgctcttccgatctnnnnnngtnnnnnnnnnnnnnnnntaacatggg

SEQ ID NO: 156 - DNA, 57 bp, synthetic construct
  misc_feature 1..54: note = DNA
  misc_feature 55..57: note = RNA
  source 1..57: mol_type = other DNA
ctacacgacgctcttccgatctnnnnnngtnnnnnnnnnnnnnnnncgtaacatggg

SEQ ID NO: 157 - DNA, 59 bp, synthetic construct
  misc_feature 1..56: note = DNA
  misc_feature 57..59: note = RNA
  source 1..59: mol_type = other DNA
ctacacgacgctcttccgatctnnnnnngtnnnnnnnnnnnnnnnnaccgtaacatggg

SEQ ID NO: 158 - DNA, 71 bp, synthetic construct
  misc_feature 1..68: note = DNA
  misc_feature 69..71: note = RNA
  source 1..71: mol_type = other DNA
ctacacgacgctcttccgatctnnnnnngtnnnnnnnnnnnnnnnnacacaagaggcacgcgtaacatggg

SEQ ID NO: 159 - DNA, 10 bp, synthetic construct
  source 1..10: mol_type = other DNA
tttcttatat

SEQ ID NO: 160 - DNA, 20 bp, synthetic construct
  source 1..20: mol_type = other DNA
acttgtccagcctaacctgc

SEQ ID NO: 161 - DNA, 20 bp, synthetic construct
  source 1..20: mol_type = other DNA
ttaccctgggaggaaccaga

SEQ ID NO: 162 - DNA, 20 bp, synthetic construct
  source 1..20: mol_type = other DNA
tttcaggccacaactccctt

SEQ ID NO: 163 - DNA, 20 bp, synthetic construct
  source 1..20: mol_type = other DNA
cagacagaccatgatgcggg

SEQ ID NO: 164 - DNA, 20 bp, synthetic construct
  source 1..20: mol_type = other DNA
gccacaactcccttttctgg

SEQ ID NO: 165 - DNA, 20 bp, synthetic construct
  source 1..20: mol_type = other DNA
agtctctcagctggtacacg

SEQ ID NO: 166 - DNA, 20 bp, synthetic construct
  source 1..20: mol_type = other DNA
tctgatggctcaaacacagc

SEQ ID NO: 167 - DNA, 16 bp, synthetic construct
  source 1..16: mol_type = other DNA
aaaaaaaaaaaaaaaa

SEQ ID NO: 168 - DNA, 11 bp, synthetic construct
  source 1..11: mol_type = other DNA
aaaaaaaaaaa

SEQ ID NO: 169 - DNA, 11 bp, synthetic construct
  source 1..11: mol_type = other DNA
ttttttttttt

SEQ ID NO: 170 - DNA, 21 bp, synthetic construct
  source 1..21: mol_type = other DNA
aaaaaaaaaaaaaaaaaaaaa